European Patent Application EP 4 674 981 A2, published January 7, 2026. Title: Single-Molecule Phenotyping and Sequencing of Nucleic Acid Molecules. Applicant: Oxford University Innovation Limited. Application EP. The sequence listing filed with the application follows.

SEQUENCE LISTING (24 sequences)

SEQ ID NO: 1 - DNA, 22 bp, unidentified
  source 1..22: mol_type = unassigned DNA
aaatgtgatctagatcacattt

SEQ ID NO: 2 - DNA, 78 bp, unidentified
  source 1..78: mol_type = unassigned DNA
ctgctgcctcaggctcataagagcctgaggcagcagattatcgacggtggatgtatggtaatgggacgaagaatgagg

SEQ ID NO: 3 - DNA, 27 bp, unidentified
  source 1..27: mol_type = unassigned DNA
cctcattcttcgtcccattaccataca

SEQ ID NO: 4 - DNA, 65 bp, unidentified
  source 1..65: mol_type = unassigned DNA
cagtcaagagcctgaggcagcagattatcgacggtggatgtatggtaatgggacgaagaatgagg

SEQ ID NO: 5 - DNA, 29 bp, unidentified
  source 1..29: mol_type = unassigned DNA
gataatctgctgcctcaggctcttgactg

SEQ ID NO: 6 - DNA, 30 bp, unidentified
  source 1..30: mol_type = unassigned DNA
cgataatctgctgcctcaggctcttgactg

SEQ ID NO: 7 - DNA, 32 bp, unidentified
  source 1..32: mol_type = unassigned DNA
gtcgataatctgctgcctcaggctcttgactg

SEQ ID NO: 8 - DNA, 65 bp, unidentified
  source 1..65: mol_type = unassigned DNA
cagtcaagagcctgaggcagcagattatcgacggaggatgtatggtaatgggacgaagaatgagg

SEQ ID NO: 9 - DNA, 31 bp, unidentified
  source 1..31: mol_type = unassigned DNA
tcgataatctgctgcctcaggctcttgactg

SEQ ID NO: 10 - DNA, 65 bp, unidentified
  source 1..65: mol_type = unassigned DNA
cagtcaagagcctgaggcagcagattatcgaataatattgtatggtaatgggacgaagaatgagg

SEQ ID NO: 11 - DNA, 25 bp, unidentified
  source 1..25: mol_type = unassigned DNA
atctgctgcctcaggctcttgactg

SEQ ID NO: 12 - DNA, 12 bp, unidentified
  source 1..12: mol_type = unassigned DNA
tccaccgtcgat

SEQ ID NO: 13-14 - skipped (2 entries)

SEQ ID NO: 15 - DNA, 45 bp, unidentified
  source 1..45: mol_type = unassigned DNA
taaatctaaagtaacataaggtaacataacgtaagctcattcgcg

SEQ ID NO: 16 - DNA, 45 bp, unidentified
  source 1..45: mol_type = unassigned DNA
cgcgaatgagcttacgttatgttaccttatgttactttagattta

SEQ ID NO: 17 - DNA, 73 bp, unidentified
  source 1..73: mol_type = unassigned DNA
cccactgccgaatgtgagttagctcactcacgaaaaaccactgtcgaaaaagctctacgggctctggcgtcgg

SEQ ID NO: 18 - DNA, 68 bp, unidentified
  source 1..68: mol_type = unassigned DNA
ccgacgccagagcccgtagagccgacagtggcgtgagtgagctaactcacattcgaaaaagcagtggg

SEQ ID NO: 19 - DNA, 49 bp, unidentified
  source 1..49: mol_type = unassigned DNA
gtgcctaaaatgtgatctagatcacatttattgcgtagagctcactgcc

SEQ ID NO: 20 - DNA, 49 bp, unidentified
  source 1..49: mol_type = unassigned DNA
ggcagtgagctctacgcaataaatgtgatctagatcacattttaggcac

SEQ ID NO: 21 - DNA, 49 bp, unidentified
  source 1..49: mol_type = unassigned DNA
gtgcctaaaatgtgatctagatcagatttattgcgtagagctcactgcc

SEQ ID NO: 22 - DNA, 49 bp, unidentified
  source 1..49: mol_type = unassigned DNA
ggcagtgagctctacgcaataaatctgatctagatcacattttaggcac

SEQ ID NO: 23 - DNA, 20 bp, unidentified
  source 1..20: mol_type = unassigned DNA
ggcagtgagctctacgcaat

SEQ ID NO: 24 - DNA, 20 bp, unidentified
  source 1..20: mol_type = unassigned DNA
ctagatcacattttaggcac